European Patent Application EP 4 389 222 A2, published June 26, 2024. Title: METHODS AND COMPOSITIONS FOR THE TREATMENT OF HEPATITIS B INFECTION. Applicant: CLEARB THERAPEUTICS LTD. Application EP 24166331.9, filed May 9, 2019. The sequence listing filed with the application follows.

SEQUENCE LISTING (55 sequences)

SEQ ID NO: 1 - protein, 275 aa, synthetic construct
  REGION 1..275: note = Description of Artificial Sequence: Synthetic polypeptide
MDYKDDDDKENITSGFLGPLLVLQAGFFLLTRILTIPQSLDSWWTSLNFLGGTTVCLGQNSQSPTSNHSPTSCPPTCPGYRWMCLRRFIIFLFILLLCLIFLLVLLDYQGMLPVCPLIPGSSTTSTGPCRTCMTTGSGSPCKTCTTPGSGSPCKTCTTPGSGSPCKTCTTPGSGSTGQGTSMYPSCCCTKPSDGNCTCIPIPSSWAFGKFLWEWASARFSWLSLLVPFVQWFVGLSPTVWLSVIWMMWYWGPSLYSILSPFLPLLPIFFCLWVYI

SEQ ID NO: 2 - protein, 275 aa, synthetic construct
  REGION 1..275: note = Description of Artificial Sequence: Synthetic polypeptide
MDYKDDDDKENITSGFLGPLLVLQAGFFLLTRILTIPQSLDSWWTSLNFLGGTTVCLGQNSQSPTSNHSPTSCPPTCPGYRWMCLRRFIIFLFILLLCLIFLLVLLDYQGMLPVCPLIPGSSTTSTGPCRTCMTTGSGSPCRTCTTPGSGSPCRTCTTPGSGSPCRTCTTPGSGSTGQGTSMYPSCCCTKPSDGNCTCIPIPSSWAFGKFLWEWASARFSWLSLLVPFVQWFVGLSPTVWLSVIWMMWYWGPSLYSILSPFLPLLPIFFCLWVYI

SEQ ID NO: 3 - protein, 278 aa, synthetic construct
  REGION 1..278: note = Description of Artificial Sequence: Synthetic polypeptide
MDYKDDDDKENITSGFLGPLLVLQAGFFLLTRILTIPQSLDSWWTSLNFLGGTTVCLGQNSQSPTSNHSPTSCPPTCPGYRWMCLRRFIIFLFILLLCLIFLLVLLDYQGMLPVCPLIPGSSTTSTGPCRTCMTTGSGSCTKPTDGNCGSGSCTKPTDGNCGSGSCTKPTDGNCGSGSTGQGTSMYPSCCCTKPSDGNCTCIPIPSSWAFGKFLWEWASARFSWLSLLVPFVQWFVGLSPTVWLSVIWMMWYWGPSLYSILSPFLPLLPIFFCLWVYI

SEQ ID NO: 4 - protein, 279 aa, synthetic construct
  REGION 1..279: note = Description of Artificial Sequence: Synthetic polypeptide
MDYKDDDDKENITSGFLGPLLVLQAGFFLLTRILTIPQSLDSWWTSLNFLGGTTVCLGQNSQSPTSNHSPTSCPPTCPGYRWMCLRRFIIFLFILLLCLIFLLVLLDYQGMLPVCPLIPGSSTTSTGPCRTCMTTGSGSCKTCTTPAQGNSMFPSGSGSCKTCTTPAQGNSMFPSGSGSTGQGTSMYPSCCCTKPSDGNCTCIPIPSSWAFGKFLWEWASARFSWLSLLVPFVQWFVGLSPTVWLSVIWMMWYWGPSLYSILSPFLPLLPIFFCLWVYI

SEQ ID NO: 5 - protein, 260 aa, synthetic construct
  REGION 1..260: note = Description of Artificial Sequence: Synthetic polypeptide
MDYKDDDDKENITSGFLGPLLVLQAGFFLLTRILTIPQSLDSWWTSLNFLGGTTVCLGQNSQSPTSNHSPTSCPPTCPGYRWMCLRRFIIFLFILLLCLIFLLVLLDYQGMLPVCPLIPGSSTTSTGPCRTCMTTGQGTSMYPSCCCTKPSDGNCGSGSCTKPTDGNCGSGSCTKPTDGNCTCIPIPSSWAFGKFLWEWASARFSWLSLLVPFVQWFVGLSPTVWLSVIWMMWYWGPSLYSILSPFLPLLPIFFCLWVYI

SEQ ID NO: 6 - protein, 284 aa, synthetic construct
  REGION 1..284: note = Description of Artificial Sequence: Synthetic polypeptide
MDYKDDDDKENITSGFLGPLLVLQAGFFLLTRILTIPQSLDSWWTSLNFLGGTTVCLGQNSQSPTSNHSPTSCPPTCPGYRWMCLRRFIIFLFILLLCLIFLLVLLDYQGMLPVCPLIPGSSTTSTGPCKTCTTPGSGSPCKTCTTPGSGSPCRTCMTTAQGTSMYPSCCCTKPSDGNCGSGSCTKPTDGNCGSGSCTKPTDGNCTCIPIPSSWAFGKFLWEWASARFSWLSLLVPFVQWFVGLSPTVWLSVIWMMWYWGPSLYSILSPFLPLLPIFFCLWVYI

SEQ ID NO: 7 - protein, 277 aa, synthetic construct
  REGION 1..277: note = Description of Artificial Sequence: Synthetic polypeptide
MDYKDDDDKENITSGFLGPLLVLQAGFFLLTRILTIPQSLDSWWTSLNFLGGTTVCLGQNSQSPTSNHSPTSCPPTCPGYRWMCLRRFIIFLFILLLCLIFLLVLLDYQGMLPVCPLIPGSSTTSTGPCKTCTTPAQGNSMFPSCGSGSCKTCTTPAQGNSMFPSCGSGSPCRTCMTTAQGTSMYPSCCCTKPSDGNCTCIPIPSSWAFGKFLWEWASARFSWLSLLVPFVQWFVGLSPTVWLSVIWMMWYWGPSLYSILSPFLPLLPIFFCLWVYI

SEQ ID NO: 8 - protein, 266 aa, synthetic construct
  REGION 1..266: note = Description of Artificial Sequence: Synthetic polypeptide
MDYKDDDDKENITSGFLGPLLVLQAGFFLLTRILTIPQSLDSWWTSLNFLGGTTVCLGQNSQSPTSNHSPTSCPPTCPGYRWMCLRRFIIFLFILLLCLIFLLVLLDYQGMLPVCPLIPGSSTTSTGPCRTCMTTAQGTSMYPSCCCTKPSDGNCGSGSPCKTCTTPAQGNSMFPSCCCTKPTDGNCTCIPIPSSWAFGKFLWEWASARFSWLSLLVPFVQWFVGLSPTVWLSVIWMMWYWGPSLYSILSPFLPLLPIFFCLWVYI

SEQ ID NO: 9 - DNA, 846 bp, synthetic construct
  misc_feature 1..846: note = Description of Artificial Sequence: Synthetic polynucleotide
  source 1..846: mol_type = other DNA
gagctcgccaccatggactataaagacgacgatgacaaagagaacatcacatcaggattcctaggaccccttctcgtgttacaggcggggtttttcttgttgacaagaatcctcacaataccgcagagtctagactcgtggtggacttctctcaattttctagggggaactaccgtgtgtcttggccaaaattcgcagtccccaacctccaatcactcaccaacctcttgtcctccaacttgtcctggttatcgctggatgtgtctgcggcgttttatcatcttcctcttcatcctgctgctatgcctcatcttcttgttggttcttctggactatcaaggtatgttgcccgtttgtcctctaattccaggatcctcaacaaccagcacgggaccatgccggacctgcatgactaccggttccggttcaccctgcaaaacctgtactaccccaggttccggatcaccctgcaaaacctgtactaccccaggttccggatcaccctgcaaaacctgtactaccccaggttccggatcaaccggtcaaggaacctctatgtatccctcctgttgctgtaccaaaccttcggacggaaattgcacctgtattcccatcccatcatcctgggctttcggaaaattcctatgggagtgggcctcagcccgtttctcctggctcagtttactagtgccatttgttcagtggttcgtagggctttcccccactgtttggctttcagttatatggatgatgtggtattgggggccaagtctgtacagcatcttgagtccctttttaccgctgttaccaattttcttttgtctttgggtatacatttaactcgag

SEQ ID NO: 10 - DNA, 846 bp, synthetic construct
  misc_feature 1..846: note = Description of Artificial Sequence: Synthetic polynucleotide
  source 1..846: mol_type = other DNA
gagctcgccaccatggactataaagacgacgatgacaaagagaacatcacatcaggattcctaggaccccttctcgtgttacaggcggggtttttcttgttgacaagaatcctcacaataccgcagagtctagactcgtggtggacttctctcaattttctagggggaactaccgtgtgtcttggccaaaattcgcagtccccaacctccaatcactcaccaacctcttgtcctccaacttgtcctggttatcgctggatgtgtctgcggcgttttatcatcttcctcttcatcctgctgctatgcctcatcttcttgttggttcttctggactatcaaggtatgttgcccgtttgtcctctaattccaggatcctcaacaaccagcacgggaccatgccggacctgcatgactaccggttccggttcaccctgccggacctgtactaccccaggttccggatcaccctgccggacctgtactaccccaggttccggatcaccctgccggacctgtactaccccaggttccggatcaaccggtcaaggaacctctatgtatccctcctgttgctgtaccaaaccttcggacggaaattgcacctgtattcccatcccatcatcctgggctttcggaaaattcctatgggagtgggcctcagcccgtttctcctggctcagtttactagtgccatttgttcagtggttcgtagggctttcccccactgtttggctttcagttatatggatgatgtggtattgggggccaagtctgtacagcatcttgagtccctttttaccgctgttaccaattttcttttgtctttgggtatacatttaactcgag

SEQ ID NO: 11 - DNA, 855 bp, synthetic construct
  misc_feature 1..855: note = Description of Artificial Sequence: Synthetic polynucleotide
  source 1..855: mol_type = other DNA
gagctcgccaccatggactataaagacgacgatgacaaagagaacatcacatcaggattcctaggaccccttctcgtgttacaggcggggtttttcttgttgacaagaatcctcacaataccgcagagtctagactcgtggtggacttctctcaattttctagggggaactaccgtgtgtcttggccaaaattcgcagtccccaacctccaatcactcaccaacctcttgtcctccaacttgtcctggttatcgctggatgtgtctgcggcgttttatcatcttcctcttcatcctgctgctatgcctcatcttcttgttggttcttctggactatcaaggtatgttgcccgtttgtcctctaattccaggatcctcaacaaccagcacgggaccatgccggacctgcatgactaccggttccggttcatgtactaaaccaaccgacggaaattgcggttccggttcatgtactaaaccaaccgacggaaattgcggttccggttcatgtactaaaccaaccgacggaaattgcggttccggttcaaccggtcaaggaacctctatgtatccctcctgttgctgtaccaaaccttcggacggaaattgcacctgtattcccatcccatcatcctgggctttcggaaaattcctatgggagtgggcctcagcccgtttctcctggctcagtttactagtgccatttgttcagtggttcgtagggctttcccccactgtttggctttcagttatatggatgatgtggtattgggggccaagtctgtacagcatcttgagtccctttttaccgctgttaccaattttcttttgtctttgggtatacatttaactcgag

SEQ ID NO: 12 - DNA, 858 bp, synthetic construct
  misc_feature 1..858: note = Description of Artificial Sequence: Synthetic polynucleotide
  source 1..858: mol_type = other DNA
gagctcgccaccatggactataaagacgacgatgacaaagagaacatcacatcaggattcctaggaccccttctcgtgttacaggcggggtttttcttgttgacaagaatcctcacaataccgcagagtctagactcgtggtggacttctctcaattttctagggggaactaccgtgtgtcttggccaaaattcgcagtccccaacctccaatcactcaccaacctcttgtcctccaacttgtcctggttatcgctggatgtgtctgcggcgttttatcatcttcctcttcatcctgctgctatgcctcatcttcttgttggttcttctggactatcaaggtatgttgcccgtttgtcctctaattccaggatcctcaacaaccagcacgggaccatgccggacctgcatgactaccggttccggttcatgtaaaacttgcactaccccagctcaaggaaattctatgttcccttccggttccggatcatgtaaaacttgcactaccccagctcaaggaaattctatgttcccttccggttccggatcaaccggtcaaggaacctctatgtatccctcctgttgctgtaccaaaccttcggacggaaattgcacctgtattcccatcccatcatcctgggctttcggaaaattcctatgggagtgggcctcagcccgtttctcctggctcagtttactagtgccatttgttcagtggttcgtagggctttcccccactgtttggctttcagttatatggatgatgtggtattgggggccaagtctgtacagcatcttgagtccctttttaccgctgttaccaattttcttttgtctttgggtatacatttaactcgag

SEQ ID NO: 13 - DNA, 801 bp, synthetic construct
  misc_feature 1..801: note = Description of Artificial Sequence: Synthetic polynucleotide
  source 1..801: mol_type = other DNA
gagctcgccaccatggactataaagacgacgatgacaaagagaacatcacatcaggattcctaggaccccttctcgtgttacaggcggggtttttcttgttgacaagaatcctcacaataccgcagagtctagactcgtggtggacttctctcaattttctagggggaactaccgtgtgtcttggccaaaattcgcagtccccaacctccaatcactcaccaacctcttgtcctccaacttgtcctggttatcgctggatgtgtctgcggcgttttatcatcttcctcttcatcctgctgctatgcctcatcttcttgttggttcttctggactatcaaggtatgttgcccgtttgtcctctaattccaggatcctcaacaaccagcacgggaccatgccggacctgcatgactaccggtcaaggaacctctatgtatccctcctgttgctgtaccaaaccttcggacggaaattgcggttccggttcatgtactaaaccaaccgacggaaattgcggttccggttcatgtactaaaccaaccgacggaaattgcacctgtattcccatcccatcatcctgggctttcggaaaattcctatgggagtgggcctcagcccgtttctcctggctcagtttactagtgccatttgttcagtggttcgtagggctttcccccactgtttggctttcagttatatggatgatgtggtattgggggccaagtctgtacagcatcttgagtccctttttaccgctgttaccaattttcttttgtctttgggtatacatttaactcgag

SEQ ID NO: 14 - DNA, 873 bp, synthetic construct
  misc_feature 1..873: note = Description of Artificial Sequence: Synthetic polynucleotide
  source 1..873: mol_type = other DNA
gagctcgccaccatggactataaagacgacgatgacaaagagaacatcacatcaggattcctaggaccccttctcgtgttacaggcggggtttttcttgttgacaagaatcctcacaataccgcagagtctagactcgtggtggacttctctcaattttctagggggaactaccgtgtgtcttggccaaaattcgcagtccccaacctccaatcactcaccaacctcttgtcctccaacttgtcctggttatcgctggatgtgtctgcggcgttttatcatcttcctcttcatcctgctgctatgcctcatcttcttgttggttcttctggactatcaaggtatgttgcccgtttgtcctctaattccaggatcctcaacaaccagcacgggaccatgcaaaacctgtactaccccaggttccggatcaccatgcaaaacctgtactaccccaggttccggatcaccatgccggacctgcatgactactgctcaaggaacctctatgtatccctcctgttgctgtaccaaaccttcggacggaaattgcggttccggttcatgtactaaaccaaccgacggaaattgcggttccggttcatgtactaaaccaaccgacggaaattgcacctgtattcccatcccatcatcctgggctttcggaaaattcctatgggagtgggcctcagcccgtttctcctggctcagtttactagtgccatttgttcagtggttcgtagggctttcccccactgtttggctttcagttatatggatgatgtggtattgggggccaagtctgtacagcatcttgagtccctttttaccgctgttaccaattttcttttgtctttgggtatacatttaactcgag

SEQ ID NO: 15 - DNA, 852 bp, synthetic construct
  misc_feature 1..852: note = Description of Artificial Sequence: Synthetic polynucleotide
  source 1..852: mol_type = other DNA
gagctcgccaccatggactataaagacgacgatgacaaagagaacatcacatcaggattcctaggaccccttctcgtgttacaggcggggtttttcttgttgacaagaatcctcacaataccgcagagtctagactcgtggtggacttctctcaattttctagggggaactaccgtgtgtcttggccaaaattcgcagtccccaacctccaatcactcaccaacctcttgtcctccaacttgtcctggttatcgctggatgtgtctgcggcgttttatcatcttcctcttcatcctgctgctatgcctcatcttcttgttggttcttctggactatcaaggtatgttgcccgtttgtcctctaattccaggatcctcaacaaccagcacgggaccatgcaaaacctgcaccactccagcgcaaggaaattctatgtttccctcctgtggttccggttcatgcaaaacctgcaccactccagcgcaaggaaattctatgtttccctcctgtggttccggttcaccatgccggacctgcatgactactgctcaaggaacctctatgtatccctcctgttgctgtaccaaaccttcggacggaaattgcacctgtattcccatcccatcatcctgggctttcggaaaattcctatgggagtgggcctcagcccgtttctcctggctcagtttactagtgccatttgttcagtggttcgtagggctttcccccactgtttggctttcagttatatggatgatgtggtattgggggccaagtctgtacagcatcttgagtccctttttaccgctgttaccaattttcttttgtctttgggtatacatttaactcgag

SEQ ID NO: 16 - DNA, 819 bp, synthetic construct
  misc_feature 1..819: note = Description of Artificial Sequence: Synthetic polynucleotide
  source 1..819: mol_type = other DNA
gagctcgccaccatggactataaagacgacgatgacaaagagaacatcacatcaggattcctaggaccccttctcgtgttacaggcggggtttttcttgttgacaagaatcctcacaataccgcagagtctagactcgtggtggacttctctcaattttctagggggaactaccgtgtgtcttggccaaaattcgcagtccccaacctccaatcactcaccaacctcttgtcctccaacttgtcctggttatcgctggatgtgtctgcggcgttttatcatcttcctcttcatcctgctgctatgcctcatcttcttgttggttcttctggactatcaaggtatgttgcccgtttgtcctctaattccaggatcctcaacaaccagcacgggaccatgccggacctgcatgactactgctcaaggaacctctatgtatccctcctgttgctgtaccaaaccttcggacggaaattgcggttccggttcaccatgcaaaacctgtactaccccagcgcaaggaaattctatgtttccctcctgctgttgcactaaaccaaccgacggaaattgcacctgtattcccatcccatcatcctgggctttcggaaaattcctatgggagtgggcctcagcccgtttctcctggctcagtttactagtgccatttgttcagtggttcgtagggctttcccccactgtttggctttcagttatatggatgatgtggtattgggggccaagtctgtacagcatcttgagtccctttttaccgctgttaccaattttcttttgtctttgggtatacatttaactcgag

SEQ ID NO: 17 - protein, 15 aa, synthetic construct
  REGION 1..15: note = Description of Artificial Sequence: Synthetic peptide
TCTTPAQGNSMFPSC

SEQ ID NO: 18 - protein, 15 aa, synthetic construct
  REGION 1..15: note = Description of Artificial Sequence: Synthetic peptide
TCTIPAQGTSMFPSC

SEQ ID NO: 19 - protein, 15 aa, synthetic construct
  REGION 1..15: note = Description of Artificial Sequence: Synthetic peptide
TCTTPAQGTSMFPSC

SEQ ID NO: 20 - protein, 10 aa, synthetic construct
  REGION 1..10: note = Description of Artificial Sequence: Synthetic peptide
CTKPTDGNCT

SEQ ID NO: 21 - protein, 10 aa, synthetic construct
  REGION 1..10: note = Description of Artificial Sequence: Synthetic peptide
CTKPSDGNCT

SEQ ID NO: 22 - DNA, 681 bp, synthetic construct
  misc_feature 1..681: note = Description of Artificial Sequence: Synthetic polynucleotide
  source 1..681: mol_type = other DNA
atggagaacatcacatcaggattcctaggaccccttctcgtgttacaggcggggtttttcttgttgacaagaatcctcacaataccgcagagtctagactcgtggtggacttctctcaattttctagggggaactaccgtgtgtcttggccaaaattcgcagtccccaacctccaatcactcaccaacctcttgtcctccaacttgtcctggttatcgctggatgtgtctgcggcgttttatcatcttcctcttcatcctgctgctatgcctcatcttcttgttggttcttctggactatcaaggtatgttgcccgtttgtcctctaattccaggatcctcaacaaccagcacgggaccatgccggacctgcatgactaccggtcaaggaacctctatgtatccctcctgttgctgtaccaaaccttcggacggaaattgcacctgtattcccatcccatcatcctgggctttcggaaaattcctatgggagtgggcctcagcccgtttctcctggctcagtttactagtgccatttgttcagtggttcgtagggctttcccccactgtttggctttcagttatatggatgatgtggtattgggggccaagtctgtacagcatcttgagtccctttttaccgctgttaccaattttcttttgtctttgggtatacatttaa

SEQ ID NO: 23 - DNA, 705 bp, synthetic construct
  misc_feature 1..705: note = Description of Artificial Sequence: Synthetic polynucleotide
  source 1..705: mol_type = other DNA
atggactataaagacgacgatgacaaagagaacatcacatcaggattcctaggaccccttctcgtgttacaggcggggtttttcttgttgacaagaatcctcacaataccgcagagtctagactcgtggtggacttctctcaattttctagggggaactaccgtgtgtcttggccaaaattcgcagtccccaacctccaatcactcaccaacctcttgtcctccaacttgtcctggttatcgctggatgtgtctgcggcgttttatcatcttcctcttcatcctgctgctatgcctcatcttcttgttggttcttctggactatcaaggtatgttgcccgtttgtcctctaattccaggatcctcaacaaccagcacgggaccatgccggacctgcatgactaccggtcaaggaacctctatgtatccctcctgttgctgtaccaaaccttcggacggaaattgcacctgtattcccatcccatcatcctgggctttcggaaaattcctatgggagtgggcctcagcccgtttctcctggctcagtttactagtgccatttgttcagtggttcgtagggctttcccccactgtttggctttcagttatatggatgatgtggtattgggggccaagtctgtacagcatcttgagtccctttttaccgctgttaccaattttcttttgtctttgggtatacatttaa

SEQ ID NO: 24 - protein, 16 aa, synthetic construct
  REGION 1..16: note = Description of Artificial Sequence: Synthetic peptide
  VARIANT 2: note = K or R
  VARIANT 5: note = T or M
  VARIANT 6: note = T or I
  VARIANT 7: note = P, T, or L
  VARIANT 8: note = A or V
  VARIANT 11: note = N or T
  VARIANT 14: note = F or Y
CXTCXXXXQGXSMXPC

SEQ ID NO: 25 - protein, 8 aa, synthetic construct
  REGION 1..8: note = Description of Artificial Sequence: Synthetic peptide
  VARIANT 3: note = K or R
  VARIANT 6: note = T or M
  VARIANT 7: note = T, I, S, or A
  VARIANT 8: note = P, T, or L
PCXTCXXX

SEQ ID NO: 26 - protein, 12 aa, synthetic construct
  REGION 1..12: note = Description of Artificial Sequence: Synthetic peptide
  VARIANT 7: note = T or S
  VARIANT 12: note = T or S
CCCTKPXDGNCX

SEQ ID NO: 27 - protein, 17 aa, synthetic construct
  REGION 1..17: note = Description of Artificial Sequence: Synthetic peptide
CKTCTTPAQGNSMFPSC

SEQ ID NO: 28 - protein, 8 aa, synthetic construct
  REGION 1..8: note = Description of Artificial Sequence: Synthetic peptide
PCKTCTTP

SEQ ID NO: 29 - protein, 12 aa, synthetic construct
  REGION 1..12: note = Description of Artificial Sequence: Synthetic peptide
CCCTKPTDGNCT

SEQ ID NO: 30 - protein, 17 aa, synthetic construct
  REGION 1..17: note = Description of Artificial Sequence: Synthetic peptide
CKTCTIPAQGTSMFPSC

SEQ ID NO: 31 - protein, 11 aa, synthetic construct
  REGION 1..11: note = Description of Artificial Sequence: Synthetic peptide
CCTKPSDGNCT

SEQ ID NO: 32 - protein, 17 aa, synthetic construct
  REGION 1..17: note = Description of Artificial Sequence: Synthetic peptide
CRTCTTPAQGTSMFPSC

SEQ ID NO: 33 - protein, 8 aa, synthetic construct
  REGION 1..8: note = Description of Artificial Sequence: Synthetic peptide
PCRTCTTP

SEQ ID NO: 34 - protein, 9 aa, synthetic construct
  REGION 1..9: note = Description of Artificial Sequence: Synthetic peptide
CTKPTDGNC

SEQ ID NO: 35 - protein, 16 aa, synthetic construct
  REGION 1..16: note = Description of Artificial Sequence: Synthetic peptide
CKTCTTPAQGNSMFPS

SEQ ID NO: 36 - protein, 10 aa, synthetic construct
  REGION 1..10: note = Description of Artificial Sequence: Synthetic peptide
  VARIANT 5: note = T or S
CTKPXTDGNC

SEQ ID NO: 37 - protein, 8 aa, synthetic construct
  REGION 1..8: note = Description of Artificial Sequence: Synthetic peptide
  VARIANT 3: note = K or R
  VARIANT 6: note = T or M
PCXTCXTP

SEQ ID NO: 38 - protein, 16 aa, synthetic construct
  REGION 1..16: note = Description of Artificial Sequence: Synthetic peptide
  VARIANT 2: note = K or R
  VARIANT 5: note = T or M
  VARIANT 7: note = P or T
  VARIANT 11: note = N or T
  VARIANT 14: note = F or Y
CXTCXTXAQGXSMXPS

SEQ ID NO: 39 - protein, 28 aa, synthetic construct
  REGION 1..28: note = Description of Artificial Sequence: Synthetic peptide
PCRTCMTTAQGTSMYPSCCCTKPSDGNC

SEQ ID NO: 40 - protein, 28 aa, synthetic construct
  REGION 1..28: note = Description of Artificial Sequence: Synthetic peptide
PCKTCTTPAQGNSMFPSCCCTKPTDGNC

SEQ ID NO: 41 - protein, 46 aa, synthetic construct
  REGION 1..46: note = Description of Artificial Sequence: Synthetic polypeptide
MTTGSGSPCKTCTTPGSGSPCKTCTTPGSGSPCKTCTTPGSGSTGQ

SEQ ID NO: 42 - protein, 46 aa, synthetic construct
  REGION 1..46: note = Description of Artificial Sequence: Synthetic polypeptide
MTTGSGSPCRTCTTPGSGSPCRTCTTPGSGSPCRTCTTPGSGSTGQ

SEQ ID NO: 43 - protein, 49 aa, synthetic construct
  REGION 1..49: note = Description of Artificial Sequence: Synthetic polypeptide
MTTGSGSCTKPTDGNCGSGSCTKPTDGNCGSGSCTKPTDGNCGSGSTGQ

SEQ ID NO: 44 - protein, 49 aa, synthetic construct
  REGION 1..49: note = Description of Artificial Sequence: Synthetic polypeptide
MTTGSGSCKTCTTPAQGNSMFPSGSGSCKTCTTPAQGNSMFPSGSGSTG

SEQ ID NO: 45 - protein, 41 aa, synthetic construct
  REGION 1..41: note = Description of Artificial Sequence: Synthetic polypeptide
CCCTKPSDGNCGSGSCTKPTDGNCGSGSCTKPTDGNCTCIP

SEQ ID NO: 46 - protein, 39 aa, synthetic construct
  REGION 1..39: note = Description of Artificial Sequence: Synthetic polypeptide
STGPCKTCTTPGSGSPCKTCTTPGSGSPCRTCMTTAQGT

SEQ ID NO: 47 - protein, 41 aa, synthetic construct
  REGION 1..41: note = Description of Artificial Sequence: Synthetic polypeptide
SCCCTKPSDGNCGSGSCTKPTDGNCGSGSCTKPTDGNCTCI

SEQ ID NO: 48 - protein, 17 aa, synthetic construct
  REGION 1..17: note = Description of Artificial Sequence: Synthetic peptide
PCRTCMTTAQGTSMYPS

SEQ ID NO: 49 - protein, 66 aa, synthetic construct
  REGION 1..66: note = Description of Artificial Sequence: Synthetic polypeptide
TGPCKTCTTPAQGNSMFPSCGSGSCKTCTTPAQGNSMFPSCGSGSPCRTCMTTAQGTSMYPSCCCT

SEQ ID NO: 50 - protein, 226 aa, synthetic construct
  REGION 1..226: note = Description of Artificial Sequence: Synthetic polypeptide
MENITSGFLGPLLVLQAGFFLLTRILTIPQSLDSWWTSLNFLGGTTVCLGQNSQSPTSNHSPTSCPPTCPGYRWMCLRRFIIFLFILLLCLIFLLVLLDYQGMLPVCPLIPGSSTTSTGPCRTCMTTGQGTSMYPSCCCTKPSDGNCTCIPIPSSWAFGKFLWEWASARFSWLSLLVPFVQWFVGLSPTVWLSVIWMMWYWGPSLYSILSPFLPLLPIFFCLWVYI

SEQ ID NO: 51 - protein, 234 aa, synthetic construct
  REGION 1..234: note = Description of Artificial Sequence: Synthetic polypeptide
MDYKDDDDKENITSGFLGPLLVLQAGFFLLTRILTIPQSLDSWWTSLNFLGGTTVCLGQNSQSPTSNHSPTSCPPTCPGYRWMCLRRFIIFLFILLLCLIFLLVLLDYQGMLPVCPLIPGSSTTSTGPCRTCMTTGQGTSMYPSCCCTKPSDGNCTCIPIPSSWAFGKFLWEWASARFSWLSLLVPFVQWFVGLSPTVWLSVIWMMWYWGPSLYSILSPFLPLLPIFFCLWVYI

SEQ ID NO: 52 - protein, 16 aa, synthetic construct
  REGION 1..16: note = Description of Artificial Sequence: Synthetic peptide
CKTCTTPAQGNSMFPS

SEQ ID NO: 53 - protein, 4 aa, synthetic construct
  REGION 1..4: note = Description of Artificial Sequence: Synthetic peptide
GSGS

SEQ ID NO: 54 - protein, 9 aa, synthetic construct
  REGION 1..9: note = Description of Artificial Sequence: Synthetic peptide
CTKPSDGNC

SEQ ID NO: 55 - protein, 8 aa, synthetic construct
  REGION 1..8: note = Description of Artificial Sequence: Synthetic peptide
PCRTCMTT